European Patent Specification EP 3 824 089 B1, published May 28, 2025. Title: Nucleic Acid Molecules Comprising a Variant RpoC Coding Sequence. Applicant: CJ CHEILJEDANG CORPORATION. The sequence listing filed with the application follows.

SEQUENCE LISTING (51 sequences)

SEQ ID NO: 1 - DNA, 4224 bp, Artificial Sequence
  Synthetic construct modified rpoC
gtgaaagatttattaaagtttctgaaagcgcagactaaaaccgaagagtttgatgcgatcaaaattgctctggcttcgccagacatgatccgttcatggtctttcggtgaagttaaaaagccggaaaccatcaactactgtacgttcaaaccagaacgtgacggccttttctgcgcccgtatctttgggccggtaaaagattacgagtgcctgtgcggtaagtacaagcgcctgaaacaccgtggcgtcatctgtgagaagtgcggcgttgaagtgacccagactaaagtacgccgtgagcgtatgggccacatcgaactggcttccccgactgcgcacatctggttcctgaaatcgctgccgtcccgtatcggtctgctgctcgatatgccgctgcgcgatatcgaacgcgtactgtactttgaatcctatgtggttatcgaaggcggtatgaccaacctggaacgtcagcagatcctgactgaagagcagtatctggacgcgctggaagagttcggtgacgaattcgacgcgaagatgggggcggaagcaatccaggctctgctgaagagcatggatctggagcaagagtgcgaacagctgcgtgaagagctgaacgaaaccaactccgaaaccaagcgtaaaaagctgaccaagcgtatcaaactgctggaagcgttcgttcagtctggtaacaaaccagagtggatgatcctgaccgttctgccggtactgccgccagatctgcgtccgctggttccgctggatggtggtcgtttcgcgacttctgacctgaacgatctgtatcgtcgcgtcattaaccgtaacaaccgtctgaaacgtctgctggatctggctgcgccggacatcatcgtacgtaacgaaaaacgtatgctgcaggaagcggtagacgccctgctggataacggtcgtcgcggtcgtgcgatcaccggttctaacaagcgtcctctgaaatctttggccgacatgatcaaaggtaaacagggtcgtttccgtcagaacctgctcggtaagcgtgttgactactccggtcgttctgtaatcaccgtaggtccatacctgcgtctgcatcagtgcggtctgccgaagaaaatggcactggagctgttcaaaccgttcatctacggcaagctggaactgcgtggtcttgctaccaccattaaagctgcgaagaaaatggttgagcgcgaagaagctgtcgtttgggatatcctggacgaagttatccgcgaacacccggtactgctgaaccgtgcaccgactctgcaccgtctgggtatccaggcatttgaaccggtactgatcgaaggtaaagctatccagctgcacccgctggtttgtgcggcatataacgccgacttcgatggtgaccagatggctgttcacgtaccgctgacgctggaagcccagctggaagcgcgtgcgctgatgatgtctaccaacaacatcctgtccccggcgaacggcgaaccaatcatcgttccgtctcaggacgttgtactgggtctgtactacatgacccgtgactgtgttaacgccaaaggcgaaggcatggtgctgactggcccgaaagaagcagaacgtctgtatcgctctggtctggcttctctgcatgcgcgcgttaaagtgcgtatcaccgagtatgaaaaagatgctaacggtgaattagtagcgaaaaccagcctgaaagacacgactgttggccgtgccattctgtggatgattgtaccgaaaggtctgccttactccatcgtcaaccaggcgctgggtaaaaaagcaatctccaaaatgctgaacacctgctaccgcattctcggtctgaaaccgaccgttatttttgcggaccagatcatgtacaccggcttcgcctatgcagcgcgttctggtgcatctgttggtatcgatgacatggtcatcccggagaagaaacacgaaatcatctccgaggcagaagcagaagttgctgaaattcaggagcagttccagtctggtctggtaactgcgggcgaacgctacaacaaagttatcgatatctgggctgcggcgaacgatcgtgtatccaaagcgatgatggataacctgcaaactgaaaccgtgattaaccgtgacggtcaggaagagaagcaggtttccttcaacagcatctacatgatggccgactccggtgcgcgtggttctgcggcacagattcgtcagcttgctggtatgcgtggtctgatggcgaagccggatggctccatcatcgaaacgccaatcaccgcgaacttccgtgaaggtctgaacgtactccagtacttcatctccacccacggtgctcgtaaaggtctggcggataccgcactgaaaactgcgaactccggttacctgactcgtcgtctggttgacgtggcgcaggacctggtggttaccgaagacgattgtggtacccatgaaggtatcatgatgactccggttatcgagggtggtgacgttaaagagccgctgcgcgatcgcgtactgggtcgtgtaactgctgaagacgttctgaagccgggtactgctgatatcctcgttccgcgcaacacgctgctgcacgaacagtggtgtgacctgctggaagagaactctgtcgacgcggttaaagtacgttctgttgtatcttgtgacaccgactttggtgtatgtgcgcactgctacggtcgtgacctggcgcgtggccacatcatcaacaagggtgaagcaatcggtgttatcgcggcacagtccatcggtgaaccgggtacacagctgaccatgcgtacgttccacatcggtggtgcggcatctcgtgcggctgctgaatccagcatccaagtgaaaaacaaaggtagcatcaagctcagcaacgtgaagtcggttgtgaactccagcggtaaactggttatcacttcccgtaatactgaactgaaactgatcgacgaattcggtcgtactaaagaaagctacaaagtaccttacggtgcggtactggcgaaaggcgatggcgaacaggttgctggcggcgaaaccgttgcaaactgggacccgcacaccatgccggttatcaccgaagtaagcggttttgtacgctttactgacatgatcgacggccagaccattacgcgtcagaccgacgaactgaccggtctgtcttcgctggtggttctggattccgcagaacgtaccgcaggtggtaaagatctgcgtccggcactgaaaatcgttgatgctcagggtaacgacgttctgatcccaggtaccgatatgccagcgcagtacttcctgccgggtaaagcgattgttcagctggaagatggcgtacagatcagctctggtgacaccctggcgcgtattccgcaggaatccggcggtaccaaggacatcaccggtggtctgccgcgcgttgcggacctgttcgaagcacgtcgtccgaaagagccggcaatcctggctgaaatcagcggtatcgtttccttcggtaaagaaaccaaaggtaaacgtcgtctggttatcaccccggtagacggtagcgatccgtacgaagagatgattccgaaatggcgtcagctcaacgtgttcgaaggtgaacgtgtagaacgtggtgacgtaatttccgacggtccggaagcgccgcacgacattctgcgtctgcgtggtgttcatgctgttactcgttacatcgttaacgaagtacaggacgtataccgtctgcagggcgttaagattaacgataaacacatcgaagttatcgttcgtcagatgctgcgtaaagctaccatcgttaacgcgggtagctccgacttcctggaaggcgaacaggttgaatactctcgcgtcaagatcgcaaaccgcgaactggaagcgaacggcaaagtgggtgcaacttactcccgcgatctgctgggtatcaccaaagcgtctctggcaaccgagtccttcatctccgcggcatcgttccaggagaccactcgcgtgctgaccgaagcagccgttgcgggcaaacgcgacgaactgcgcggcctgaaagagaacgttatcgtgggtcgtctgatcccggcaggtaccggttacgcgtaccaccaggatcgtatgcgtcgccgtgctgcgggtgaagctccggctgcaccgcaggtgactgcagaagacgcatctgccagcctggcagaactgctgaacgcaggtctgggcggttctgataacgagtaa

SEQ ID NO: 2 - protein, 1407 aa, Artificial Sequence
  Synthetic construct modified RpoC
VKDLLKFLKAQTKTEEFDAIKIALASPDMIRSWSFGEVKKPETINYCTFKPERDGLFCARIFGPVKDYECLCGKYKRLKHRGVICEKCGVEVTQTKVRRERMGHIELASPTAHIWFLKSLPSRIGLLLDMPLRDIERVLYFESYVVIEGGMTNLERQQILTEEQYLDALEEFGDEFDAKMGAEAIQALLKSMDLEQECEQLREELNETNSETKRKKLTKRIKLLEAFVQSGNKPEWMILTVLPVLPPDLRPLVPLDGGRFATSDLNDLYRRVINRNNRLKRLLDLAAPDIIVRNEKRMLQEAVDALLDNGRRGRAITGSNKRPLKSLADMIKGKQGRFRQNLLGKRVDYSGRSVITVGPYLRLHQCGLPKKMALELFKPFIYGKLELRGLATTIKAAKKMVEREEAVVWDILDEVIREHPVLLNRAPTLHRLGIQAFEPVLIEGKAIQLHPLVCAAYNADFDGDQMAVHVPLTLEAQLEARALMMSTNNILSPANGEPIIVPSQDVVLGLYYMTRDCVNAKGEGMVLTGPKEAERLYRSGLASLHARVKVRITEYEKDANGELVAKTSLKDTTVGRAILWMIVPKGLPYSIVNQALGKKAISKMLNTCYRILGLKPTVIFADQIMYTGFAYAARSGASVGIDDMVIPEKKHEIISEAEAEVAEIQEQFQSGLVTAGERYNKVIDIWAAANDRVSKAMMDNLQTETVINRDGQEEKQVSFNSIYMMADSGARGSAAQIRQLAGMRGLMAKPDGSIIETPITANFREGLNVLQYFISTHGARKGLADTALKTANSGYLTRRLVDVAQDLVVTEDDCGTHEGIMMTPVIEGGDVKEPLRDRVLGRVTAEDVLKPGTADILVPRNTLLHEQWCDLLEENSVDAVKVRSVVSCDTDFGVCAHCYGRDLARGHIINKGEAIGVIAAQSIGEPGTQLTMRTFHIGGAASRAAAESSIQVKNKGSIKLSNVKSVVNSSGKLVITSRNTELKLIDEFGRTKESYKVPYGAVLAKGDGEQVAGGETVANWDPHTMPVITEVSGFVRFTDMIDGQTITRQTDELTGLSSLVVLDSAERTAGGKDLRPALKIVDAQGNDVLIPGTDMPAQYFLPGKAIVQLEDGVQISSGDTLARIPQESGGTKDITGGLPRVADLFEARRPKEPAILAEISGIVSFGKETKGKRRLVITPVDGSDPYEEMIPKWRQLNVFEGERVERGDVISDGPEAPHDILRLRGVHAVTRYIVNEVQDVYRLQGVKINDKHIEVIVRQMLRKATIVNAGSSDFLEGEQVEYSRVKIANRELEANGKVGATYSRDLLGITKASLATESFISAASFQETTRVLTEAAVAGKRDELRGLKENVIVGRLIPAGTGYAYHQDRMRRRAAGEAPAAPQVTAEDASASLAELLNAGLGGSDNE

SEQ ID NO: 3 - DNA, 36 bp, Artificial Sequence
  Synthetic construct rpoC primer
ctgcaggaattcgatcggttcttacagcctggttac

SEQ ID NO: 4 - DNA, 20 bp, Artificial Sequence
  Synthetic construct rpoC primer
gaacgtacagtagttgatgg

SEQ ID NO: 5 - DNA, 20 bp, Artificial Sequence
  Synthetic construct rpoC primer
ccatcaactactgtacgttc

SEQ ID NO: 6 - DNA, 36 bp, Artificial Sequence
  Synthetic construct rpoC primer
gtcgactagcgtgatcttggtttcggagttggtttc

SEQ ID NO: 7 - DNA, 4224 bp, Escherichia coli
gtgaaagatttattaaagtttctgaaagcgcagactaaaaccgaagagtttgatgcgatcaaaattgctctggcttcgccagacatgatccgttcatggtctttcggtgaagttaaaaagccggaaaccatcaactaccgtacgttcaaaccagaacgtgacggccttttctgcgcccgtatctttgggccggtaaaagattacgagtgcctgtgcggtaagtacaagcgcctgaaacaccgtggcgtcatctgtgagaagtgcggcgttgaagtgacccagactaaagtacgccgtgagcgtatgggccacatcgaactggcttccccgactgcgcacatctggttcctgaaatcgctgccgtcccgtatcggtctgctgctcgatatgccgctgcgcgatatcgaacgcgtactgtactttgaatcctatgtggttatcgaaggcggtatgaccaacctggaacgtcagcagatcctgactgaagagcagtatctggacgcgctggaagagttcggtgacgaattcgacgcgaagatgggggcggaagcaatccaggctctgctgaagagcatggatctggagcaagagtgcgaacagctgcgtgaagagctgaacgaaaccaactccgaaaccaagcgtaaaaagctgaccaagcgtatcaaactgctggaagcgttcgttcagtctggtaacaaaccagagtggatgatcctgaccgttctgccggtactgccgccagatctgcgtccgctggttccgctggatggtggtcgtttcgcgacttctgacctgaacgatctgtatcgtcgcgtcattaaccgtaacaaccgtctgaaacgtctgctggatctggctgcgccggacatcatcgtacgtaacgaaaaacgtatgctgcaggaagcggtagacgccctgctggataacggtcgtcgcggtcgtgcgatcaccggttctaacaagcgtcctctgaaatctttggccgacatgatcaaaggtaaacagggtcgtttccgtcagaacctgctcggtaagcgtgttgactactccggtcgttctgtaatcaccgtaggtccatacctgcgtctgcatcagtgcggtctgccgaagaaaatggcactggagctgttcaaaccgttcatctacggcaagctggaactgcgtggtcttgctaccaccattaaagctgcgaagaaaatggttgagcgcgaagaagctgtcgtttgggatatcctggacgaagttatccgcgaacacccggtactgctgaaccgtgcaccgactctgcaccgtctgggtatccaggcatttgaaccggtactgatcgaaggtaaagctatccagctgcacccgctggtttgtgcggcatataacgccgacttcgatggtgaccagatggctgttcacgtaccgctgacgctggaagcccagctggaagcgcgtgcgctgatgatgtctaccaacaacatcctgtccccggcgaacggcgaaccaatcatcgttccgtctcaggacgttgtactgggtctgtactacatgacccgtgactgtgttaacgccaaaggcgaaggcatggtgctgactggcccgaaagaagcagaacgtctgtatcgctctggtctggcttctctgcatgcgcgcgttaaagtgcgtatcaccgagtatgaaaaagatgctaacggtgaattagtagcgaaaaccagcctgaaagacacgactgttggccgtgccattctgtggatgattgtaccgaaaggtctgccttactccatcgtcaaccaggcgctgggtaaaaaagcaatctccaaaatgctgaacacctgctaccgcattctcggtctgaaaccgaccgttatttttgcggaccagatcatgtacaccggcttcgcctatgcagcgcgttctggtgcatctgttggtatcgatgacatggtcatcccggagaagaaacacgaaatcatctccgaggcagaagcagaagttgctgaaattcaggagcagttccagtctggtctggtaactgcgggcgaacgctacaacaaagttatcgatatctgggctgcggcgaacgatcgtgtatccaaagcgatgatggataacctgcaaactgaaaccgtgattaaccgtgacggtcaggaagagaagcaggtttccttcaacagcatctacatgatggccgactccggtgcgcgtggttctgcggcacagattcgtcagcttgctggtatgcgtggtctgatggcgaagccggatggctccatcatcgaaacgccaatcaccgcgaacttccgtgaaggtctgaacgtactccagtacttcatctccacccacggtgctcgtaaaggtctggcggataccgcactgaaaactgcgaactccggttacctgactcgtcgtctggttgacgtggcgcaggacctggtggttaccgaagacgattgtggtacccatgaaggtatcatgatgactccggttatcgagggtggtgacgttaaagagccgctgcgcgatcgcgtactgggtcgtgtaactgctgaagacgttctgaagccgggtactgctgatatcctcgttccgcgcaacacgctgctgcacgaacagtggtgtgacctgctggaagagaactctgtcgacgcggttaaagtacgttctgttgtatcttgtgacaccgactttggtgtatgtgcgcactgctacggtcgtgacctggcgcgtggccacatcatcaacaagggtgaagcaatcggtgttatcgcggcacagtccatcggtgaaccgggtacacagctgaccatgcgtacgttccacatcggtggtgcggcatctcgtgcggctgctgaatccagcatccaagtgaaaaacaaaggtagcatcaagctcagcaacgtgaagtcggttgtgaactccagcggtaaactggttatcacttcccgtaatactgaactgaaactgatcgacgaattcggtcgtactaaagaaagctacaaagtaccttacggtgcggtactggcgaaaggcgatggcgaacaggttgctggcggcgaaaccgttgcaaactgggacccgcacaccatgccggttatcaccgaagtaagcggttttgtacgctttactgacatgatcgacggccagaccattacgcgtcagaccgacgaactgaccggtctgtcttcgctggtggttctggattccgcagaacgtaccgcaggtggtaaagatctgcgtccggcactgaaaatcgttgatgctcagggtaacgacgttctgatcccaggtaccgatatgccagcgcagtacttcctgccgggtaaagcgattgttcagctggaagatggcgtacagatcagctctggtgacaccctggcgcgtattccgcaggaatccggcggtaccaaggacatcaccggtggtctgccgcgcgttgcggacctgttcgaagcacgtcgtccgaaagagccggcaatcctggctgaaatcagcggtatcgtttccttcggtaaagaaaccaaaggtaaacgtcgtctggttatcaccccggtagacggtagcgatccgtacgaagagatgattccgaaatggcgtcagctcaacgtgttcgaaggtgaacgtgtagaacgtggtgacgtaatttccgacggtccggaagcgccgcacgacattctgcgtctgcgtggtgttcatgctgttactcgttacatcgttaacgaagtacaggacgtataccgtctgcagggcgttaagattaacgataaacacatcgaagttatcgttcgtcagatgctgcgtaaagctaccatcgttaacgcgggtagctccgacttcctggaaggcgaacaggttgaatactctcgcgtcaagatcgcaaaccgcgaactggaagcgaacggcaaagtgggtgcaacttactcccgcgatctgctgggtatcaccaaagcgtctctggcaaccgagtccttcatctccgcggcatcgttccaggagaccactcgcgtgctgaccgaagcagccgttgcgggcaaacgcgacgaactgcgcggcctgaaagagaacgttatcgtgggtcgtctgatcccggcaggtaccggttacgcgtaccaccaggatcgtatgcgtcgccgtgctgcgggtgaagctccggctgcaccgcaggtgactgcagaagacgcatctgccagcctggcagaactgctgaacgcaggtctgggcggttctgataacgagtaa

SEQ ID NO: 8 - DNA, 20 bp, Artificial Sequence
  Synthetic construct pJSL47 primer
gagcgtccggtaaccgttgg

SEQ ID NO: 9 - DNA, 20 bp, Artificial Sequence
  Synthetic construct pJSL47 primer
gtcaggatcatccactctgg

SEQ ID NO: 10 - DNA, 20 bp, Artificial Sequence
  Synthetic construct repFIC primer
cgggtgggattgaatcagat

SEQ ID NO: 11 - DNA, 21 bp, Artificial Sequence
  Synthetic construct repFIC primer
tacgtttgccatgcgctatta

SEQ ID NO: 12 - DNA, 20 bp, Artificial Sequence
  Synthetic construct lacZ primer
ccttactgccgcctgttttg

SEQ ID NO: 13 - DNA, 20 bp, Artificial Sequence
  Synthetic construct lacZ primer
ccactggtgtgggccataat

SEQ ID NO: 14 - DNA, 2459 bp, Escherichia coli
atgtcgcagacagaaaatgcagtgacttcctcatcaggtaacaagcgtgcataccggaaaggtaaccctgttccggccagagagaggcaaagggcttctctagctcgcagaagcaacactcataaggcttttcatgcggttatccaggcccggttaaaagacaggctgagtgaactggcagatgaggaaggtattacccaggcgcagatgcttgaaaaactgattgaatcagagctgaaacgcagagcgactttgtaaatattcacattcttgcttatctcaggcgtgagtgatagattgctgatcgtttaaggaattttgtggctggccacgccataaggtggcagggaactggttctgatgtggatttacaggagccagaaaagcaaaaaccccgataatcttcatctagttttgcgacgaggagaagattaccgggatccacttaaaccgtatagccaacaattcagctatgcggggagtatagttatatgcccggaaaagttcaagacttctttctgtgctcactccttctgtgcattgtaagtgcaggatggtgtggctaatcatgaaacacattcagtaatagcgggtgggattgaatcagatcttcacattgattccagcaagtatcctcacccgttttgcagccttctccagaaaagggctcattttgactccttcaagcatctgatcttcatcagaggtttgcttgtaatagcgcatggcaaacgtaaaaataaaatcagcgcgtcgatggttagtttttatgtttccctcgtacaagtaatgtgcgcacactacatccctgatacgaacaaagttaacttatctgttaaagagctttcagtttgtagtggaggttcatacactcgtgtttggagagccctcaaaactcttgataatgatcttcatctcatcgcttttgatggaggaaccatctggttcagaccagatatgttcgaaactttacgtgtcggcccagacgagctagttgccgcccgtaggagggggaatagtgttggagggggacatggctgatctccttcaaaaatactattcacaggttaaaaacccgaatccggtgttcacaccccgtgaaggtgccggaacgctgaagttctgcgaaaaactgatggaaaaggcggtgggcttcacctcccgttttgatttcgccattcatgtggcacatgctcgttcgaagggactgcgtcggcgcatgccaccggtactgcgtcgccgggctattgatgcgctgctgcaggggctgtgttttcactatgacccgctggccaaccgcgtccagtgctccatcactacgctggccattgagtgcggactggcgacggagtctgctgccggaaaactctccatcacccgggccacccgagccttgacgttccttgcagagctgggactgattacctaccagacggaatatgatccgcttatcgggtgctacattccgaccgatatcacgttcacaccggcgctatttgccgcccttgatgtgtctgaggatgcagtggttgctgcgcgccgcagtcgtgttgaatgggaaaacagacagcgcaaaaagcagggactggataccctgggtatggatgaactgatagcgaaagcctggcgttttgtgcgtgagcgtttccgcagttaccagacagagcttaagtcccgtggaataaagcgtgcccgtgcgcgtcgtgatgcgaacagggaacgtcaggatatcgtcaccctggtgaaacggcagctgacgcgtgaaatctcggaagggcgcttcactgccaatcgtgaggcggtaaaacgcgaagtggagcgtcgtgtgaaagatcgcatgattctgtcacgtaaccgtaattacagccggctggccacagcttccccctgaaagtgacctcctctgaataatccggcccgcaccggaggcatctgcacgcctgaagcctgtcggcgaacaaaaaaacagcaccgcatacaaaaaacaacctcatcatccaccttcaggtgcatccggtccctcctgtttttgatacaaaacacgcctcacagacgaggaattttgcttatccacatttaactgcaagggacttccccataaggttacaaccgttcatgtcataaagcgccatccgccagccttacagggtgcaatgtatcttttaaacacctgtttatatctcctttaaactacttaactacattcatttaaaaagaaaacctattcactgcctgtcctgtggacagacaggtatgcacctcccaccgcaagcggcgggccccgaccggagccactttaattacaacactcagatacaaccaccagaaaaaccccggtcccgcgcagaactgaaaccacaaagccccccctcataactgaaaagcggccccgccccggcccaaagggccggaacagagtcgcttttaattatgaatgttgtaactacacagcatcatcg

SEQ ID NO: 15 - DNA, 35 bp, Artificial Sequence
  Synthetic construct repFIC primer
ttccggaagtgtgaggcggccgcacttgtgtataa

SEQ ID NO: 16 - DNA, 35 bp, Artificial Sequence
  Synthetic construct repFIC primer
gtcgacaagctttacgcggccagatctgatcaaga

SEQ ID NO: 17 - DNA, 35 bp, Artificial Sequence
  Synthetic construct kanamycin primer
atcagatctggccgcgtaaagcttgtcgacgaatt

SEQ ID NO: 18 - DNA, 35 bp, Artificial Sequence
  Synthetic construct kanamycin primer
cacaagtgcggccgcctcacacttccggaaagcgg

SEQ ID NO: 19 - DNA, 98 bp, Artificial Sequence
  Synthetic construct repFIC sequence
aagcaaaaaccccgataatcttcatctagttttgcgacaaggagaagattaccgggatccacttaaaccgtatagccaacaattcagctatgcgggga

SEQ ID NO: 20 - DNA, 20 bp, Artificial Sequence
  Synthetic construct repFIC primer
tcttctccttgtcgcaaaac

SEQ ID NO: 21 - DNA, 20 bp, Artificial Sequence
  Synthetic construct repFIC primer
gttttgcgacaaggagaaga

SEQ ID NO: 22 - DNA, 20 bp, Artificial Sequence
  Synthetic construct kanamycin primer
gcagccgattgtctgttgtg

SEQ ID NO: 23 - DNA, 20 bp, Artificial Sequence
  Synthetic construct kanamycin primer
atggattgcacgcaggttct

SEQ ID NO: 24 - DNA, 20 bp, Artificial Sequence
  Synthetic construct repFIA primer
atggctcaggcatcgtctct

SEQ ID NO: 25 - DNA, 20 bp, Artificial Sequence
  Synthetic construct repFIA primer
agaggcgcattggagttctg

SEQ ID NO: 26 - protein, 1407 aa, Escherichia coli [sequence omitted]

SEQ ID NO: 27 - protein, 1407 aa, Artificial Sequence
  Synthetic construct modified RpoC
MKDLLKFLKAQTKTEEFDAIKIALASPDMIRSWSFGEVKKPETINYCTFKPERDGLFCARIFGPVKDYECLCGKYKRLKHRGVICEKCGVEVTQTKVRRERMGHIELASPTAHIWFLKSLPSRIGLLLDMPLRDIERVLYFESYVVIEGGMTNLERQQILTEEQYLDALEEFGDEFDAKMGAEAIQALLKSMDLEQECEQLREELNETNSETKRKKLTKRIKLLEAFVQSGNKPEWMILTVLPVLPPDLRPLVPLDGGRFATSDLNDLYRRVINRNNRLKRLLDLAAPDIIVRNEKRMLQEAVDALLDNGRRGRAITGSNKRPLKSLADMIKGKQGRFRQNLLGKRVDYSGRSVITVGPYLRLHQCGLPKKMALELFKPFIYGKLELRGLATTIKAAKKMVEREEAVVWDILDEVIREHPVLLNRAPTLHRLGIQAFEPVLIEGKAIQLHPLVCAAYNADFDGDQMAVHVPLTLEAQLEARALMMSTNNILSPANGEPIIVPSQDVVLGLYYMTRDCVNAKGEGMVLTGPKEAERLYRSGLASLHARVKVRITEYEKDANGELVAKTSLKDTTVGRAILWMIVPKGLPYSIVNQALGKKAISKMLNTCYRILGLKPTVIFADQIMYTGFAYAARSGASVGIDDMVIPEKKHEIISEAEAEVAEIQEQFQSGLVTAGERYNKVIDIWAAANDRVSKAMMDNLQTETVINRDGQEEKQVSFNSIYMMADSGARGSAAQIRQLAGMRGLMAKPDGSIIETPITANFREGLNVLQYFISTHGARKGLADTALKTANSGYLTRRLVDVAQDLVVTEDDCGTHEGIMMTPVIEGGDVKEPLRDRVLGRVTAEDVLKPGTADILVPRNTLLHEQWCDLLEENSVDAVKVRSVVSCDTDFGVCAHCYGRDLARGHIINKGEAIGVIAAQSIGEPGTQLTMRTFHIGGAASRAAAESSIQVKNKGSIKLSNVKSVVNSSGKLVITSRNTELKLIDEFGRTKESYKVPYGAVLAKGDGEQVAGGETVANWDPHTMPVITEVSGFVRFTDMIDGQTITRQTDELTGLSSLVVLDSAERTAGGKDLRPALKIVDAQGNDVLIPGTDMPAQYFLPGKAIVQLEDGVQISSGDTLARIPQESGGTKDITGGLPRVADLFEARRPKEPAILAEISGIVSFGKETKGKRRLVITPVDGSDPYEEMIPKWRQLNVFEGERVERGDVISDGPEAPHDILRLRGVHAVTRYIVNEVQDVYRLQGVKINDKHIEVIVRQMLRKATIVNAGSSDFLEGEQVEYSRVKIANRELEANGKVGATYSRDLLGITKASLATESFISAASFQETTRVLTEAAVAGKRDELRGLKENVIVGRLIPAGTGYAYHQDRMRRRAAGEAPAAPQVTAEDASASLAELLNAGLGGSDNE

SEQ ID NO: 28 - protein, 9 aa, Artificial Sequence
  Synthetic construct modified RpoC N terminal domain
KPETINYCT

SEQ ID NO: 29 - protein, 7 aa, Artificial Sequence
  Synthetic construct modified RpoC central domain
NADFDGD

SEQ ID NO: 30 - protein, 6 aa, Artificial Sequence
  Synthetic construct modified RpoC C-terminal domain
SAASFQ

SEQ ID NO: 31 - protein, 25 aa, Artificial Sequence
  Synthetic construct modified RpoC N terminal domain extended
WSFGEVKKPETINYCTFKPERDGLF

SEQ ID NO: 32 - protein, 23 aa, Artificial Sequence
  Synthetic construct modified RpoC central domain extended
HPLVCAAYNADFDGDQMAVHVPL

SEQ ID NO: 33 - protein, 55 aa, Artificial Sequence
  Synthetic construct modified RpoC C-terminal domain extended
GITKASLATESFISAASFQETTRVLTEAAVAGKRDELRGLKENVIVGRLIPAGTG

SEQ ID NO: 34 - protein, 1524 aa, Thermus thermophilus
MKKEVRKVRIALASPEKIRSWSYGEVEKPETINYRTLKPERDGLFDERIFGPIKDYECACGKYKRQRFEGKVCERCGVEVTKSIVRRYRMGHIELATPAAHIWFVKDVPSKIGTLLDLSATELEQVLYFSKYIVLDPKGAILNGVPVEKRQLLTDEEYRELRYGKQETYPLPPGVDALVKDGEEVVKGQELAPGVVSRLDGVALYRFPRRVRVEYVKKERAGLRLPLAAWVEKEAYKPGEILAELPEPYLFRAEEEGVVELKELEEGAFLVLRREDEPVATYFLPVGMTPLVVHGEIVEKGQPLAEAKGLLRMPRQVRAAQVEAEEEGETVYLTLFLEWTEPKDYRVQPHMNVVVPEGARVEAGDKIVAAIDPEEEVIAEAEGVVHLHEPASILVVKARVYPFEDDVEVSTGDRVAPGDVLADGGKVKSDVYGRVEVDLVRNVVRVVESYDIDARMGAEAIQQLLKELDLEALEKELLEEMKHPSRARRAKARKRLEVVRAFLDSGNRPEWMILEAVPVLPPDLRPMVQVDGGRFATSDLNDLYRRLINRNNRLKKLLAQGAPEIIIRNEKRMLQEAVDALLDNGRRGAPVTNPGSDRPLRSLTDILSGKQGRFRQNLLGKRVDYSGRSVIVVGPQLKLHQCGLPKRMALELFKPFLLKKMEEKGIAPNVKAARRMLERQRDIKDEVWDALEEVIHGKVVLLNRAPTLHRLGIQAFQPVLVEGQSIQLHPLVCEAFNADFDGDQMAVHVPLSSFAQAEARIQMLSAHNLLSPASGEPLAKPSRDIILGLYYITQVRKEKKGAGLEFATPEEALAAHERGEVALNAPIKVAGRETSVGRLKYVFANPDEALLAVAHGIVDLQDVVTVRYMGKRLETSPGRILFARIVAEAVEDEKVAWELIQLDVPQEKNSLKDLVYQAFLRLGMEKTARLLDALKYYGFTFSTTSGITIGIDDAVIPEEKKQYLEEADRKLLQIEQAYEMGFLTDRERYDQILQLWTETTEKVTQAVFKNFEENYPFNPLYVMAQSGARGNPQQIRQLCGLRGLMQKPSGETFEVPVRSSFREGLTVLEYFISSHGARKGGADTALRTADSGYLTRKLVDVTHEIVVREADCGTTNYISVPLFQPDEVTRSLRLRKRADIEAGLYGRVLAREVEVLGVRLEEGRYLSMDDVHLLIKAAEAGEIQEVPVRSPLTCQTRYGVCQKCYGYDLSMARPVSIGEAVGIVAAQSIGEPGTQLTMRTFHTGGVAGAADITQGLPRVIELFEARRPKAKAVISEIDGVVRIEETEEKLSVFVESEGFSKEYKLPKEARLLVKDGDYVEAGQPLTRGAIDPHQLLEAKGPEAVERYLVEEIQKVYRAQGVKLHDKHIEIVVRQMMKYVEVTDPGDSRLLEGQVLEKWDVEALNERLIAEGKTPVAWKPLLMGVTKSALSTKSWLSAASFQNTTHVLTEAAIAGKKDELIGLKENVILGRLIPAGTGSDFVRFTQVVDQKTLKAIEEARKEAVEAKERPAARRGVKREQPGKQA

SEQ ID NO: 35 - protein, 1391 aa, Acetobacter pasteurianus
MNELMKILGQTGQAMTFDQIKIQLASPEQIRSWSYGEIKKPETINYRTFKPERDGLFCARIFGPIKDYECLCGKYKRMKFRGIICEKCGVEVTLAKVRRERMGHIQLASPVAHIWFLKSLPSRIGLMVDMTLKDLEKVLYFESYLVLEPGTSPLKQYSLLTEEQYLDAMDEYGDEGVEVGIGAEAIKKVLERIDCDAEKVELRQELKETTSEAKRKKLVKRLKLIEAFAESGSRPEWMILDLVPVIPPDLRPLVPLDGGRFATSDLNDLYRRVINRNNRLKRLMELRAPDIIVRNEKRMLQEAVDALFDNGRRGRAITGANKRPLKSLSDMLKGKQGRFRQNLLGKRVDYSGRSVIVVGPELKLHQCGLPKKMALELFKPFIYAKLEKYGHATTIKAAKRMVEKERPEVWDILEEVIREHPVMLNRAPTLHRLGIQAFEPVLVEGKAIQLHPLVCTAFNADFDGDQMAVHVPLSLEAQLEARVLMMSTNNILSPANGKPIIVPSQDIVLGLYYLSLETPEFKVTPDRCEYDETTGALTKEGAPSFSSIGEVEYALSAGALKLHDKIRARFQKIGADGKVTYETAVTTPGRVLIAQILPQHEAVPFSLINRQLTKKAVSDVIDTVYRHCGQKEAVIFCDRLMALGFRHAAKAGISFGKDDMIIPPEKKELVDRTAAEVKEFEQQYQDGLITAGERYNKVVDAWSRCTDEVQAAMTKEISRQEVGKQINSVWMMSHSGARGSPAQMKQLAGMRGLMAKPSGEIIEQPIIANFKEGLSVLDYFTSTHGARKGLADTALKTANSGYLTRRLVDVAQDSIIIEEDCGSERGLTVRAVMDGGEVVASLSERILGRTVASDVVVPGTGEVIVPRNHLIDEADAERIEKSGVETVHIRSVLTCDSRVGVCGRCYGRDLARGTPVNIGEAVGVIAAQSIGEPGTQLTMRTFHIGGAAQRGAEQSMIEASRDGHVVIRNRNVVHNSQNVPIVMARNCEILLSDDNGVEKARYRVPYGARLLTEEGAKVARGQKLAEWDPYTLPIITEKAGKVEYLDLIDSITLVERMDEVTGLTSKVVVDYKQAGKGVDLRPRLQLKDANGDVVKLDNGADARYFLSPETLLSVENGTEVNAGDVLARLPREGSKTRDITGGLPRVAELFEARRPKDHAIIAEMEGRVEFGKDYKSKRRVIVKNDETGEEQEYLIPKGKHISVQEGDFVEKGDPLVDGPRVPHDILKVMGVEALSDYLINEIQDVYRLQGVKINDKHIEVIVRQMLQKVEILEPGDTTYLIGETVDRIEFEAENAKCLKAGERPAQGMPVLQGITKASLQTQSFISAASFQETTRVLTEAATAGKVDKLMGLKENVIVGRLIPAGTGSVMKRLRAIAAEQDRQRVGRSAAE

SEQ ID NO: 36 - protein, 1391 aa, Neisseria gonorrhoeae
MNLLNLFNPLQTAGMEEEFDAIKIGIASPETIRSWSYGEVKKPETINYRTFKPERDGLFCAKIFGPVKDYECLCGKYKRLKFKGVTCEKCGVEVTLSKVRRERMGHIELAAPVAHIWFLKSLPSRLGMVLNMTLRDIERVLYFEAFVVTDPGMTPLQRRQLLTEDDYYNKLDEYGDDFDAKMGAEGIRELLRTLDVAGEIEILRQELESTGSDTKIKKIAKRLKVLEAFHRSGMKLEWMIMDVLPVLPPDLRPLVPLDGGRFATSDLNDLYRRVINRNNRLKRLLELHAPDIIVRNEKRMLQEAVDSLLDNGRRGKAMTGANKRPLKSLADMIKGKGGRFRQNLLGKRVDYSGRSVITVGPYLRLHQCGLPKKMALELFKPFIFHKLEKQGLASTVKAAKKLVEQEVPEVWDILEEVIREHPIMLNRAPTLHRLGIQAFEPILIEGKAIQLHPLVCAAFNADFDGDQMAVHVPLSLEAQMEARTLMLASNNVLSPANGEPIIVPSQDIVLGLYYMTRDRINAKGEGSLFADVKEVHRAYHTKQVELGTKITVRLREWVKNEAGEFEPVVNRYETTVGRALLSEILPKGLPFEYVNKALKKKEISKLINASFRLCGLRDTVIFADHLMYTGFGFAAKGGISIAVDDMEIPKEKAALLAEANAEVKEIEDQYRQGLVTNGERYNKVVDIWGRAGDKIAKAMMDNLSKQKVIDRDGNEVDQESFNSIYMMADSGARGSAAQIKQLSGMRGLMAKPDGSIIETPITSNFREGLTVLQYFIATHGARKGLADTALKTANSGYLTRRLVDVTQDLVVVEDDCGTSDGFVMKAVVQGGDVIEALRDRILGRVTASDVVDPSSGETLVEAGTLLTEKLVDMIDQSGVDEVKVRTPITCKTRHGLCAHCYGRDLARGKLVNAGEAVGVIAAQSIGEPGTQLTMRTFHIGGAASRAAAASQVEAKSNGTARFSSQMRYVANNKGELVVIGRSCEVVIHDDIGRERERHKVPYGAILLVQDGMAIKAGQTLATWDPHTRPMITEHAGMVKFENMEEGVTVAKQTDDVTGLSTLVVIDGKRRSSSASKLLRPTVKLLDENGVEICIPGTSTPVSMAFPVGAVITVREGQEIGKGDVLARIPQASSKTRDITGGLPRVAELFEARVPKDAGMLAEITGTVSFGKETKGKQRLIITDVDGVAYETLISKEKQILVHDGQVVNRGETIVDGAVDPHDILRLQGIEALARYIVQEVQEVYRLQGVKISDKHIEVIIRQMLRRVNIADAGETGFITGEQVERGDVMAANEKALEEGKEPARYENILLGITKASLSTDSFISAASFQETTRVLTEAAIMGKQDELRGLKENVIVGRLIPAGTGLTYHRSRHQQWQGVEQETAETQVTDE

SEQ ID NO: 37 - protein, 1401 aa, Legionella pneumophila
MSDLLGILKQQGQSEEFDAIKIALASPELIRSWSYGEVKKPETINYRTFKPERDGLFCAKTFGPVKDYECLCGKYKRLKHRGVICEKCGVELALAKVRRERMGHIELASPVAHIWFLKSLPSRIGLLLDMTLRDIERVLYFEAFVVVDPGMTELERGQLLNDEAYLDAMEQYGDEFDARMGAEAIRDLLRQIDLEDEIRNLREELPTTNSETKIKKITKRLKLLEAFYESGNKPEWMIMDVLPVLPPDLRPLVPLDGGRFATSDLNDLYRRVINRNNRLKRLLDLNAPDIIVRNEKRMLQESVDALLDNGRRGRAITGTNKRPLKSLADMIKGKQGRFRQNLLGKRVDYSGRSVIVVGPTLKLHQCGLPKKMALELFKPFIFSKLEFRGLATTIKAAKKMVEREESVVWDILDDVIREHPILLNRAPTLHRLGIQAFEPVLIEGKAIQLHPLVCTAYNADFDGDQMAVHVPLTLEAQLEARSLMMSTNNILSPASGEPIIVPSQDVVLGLYYLTREKVNALGEGKIYSSAQEAQNFYEAGHLDIHAKIKIRMPKEDGETGYHLVETTVGRAILAEILPKGMPFDYINRTMTKKVISKVIDSCYRKFGLKETVIFADQLMYTGFKYATRSGASIGIEDMEIPDDKSSIIEHADNEVREIESQFRSGLVTNGERYNKVIDIWSRTNELVAKSMMSKIATEEVTDAKGNKVRQESFNPIFMMADSGARGSAAQIRQLAGMRGLMAAPDGSIIETPITANFREGLNVFQYFISTHGARKGLADTALKTANSGYLTRRLVDVAQDVVITEDDCGTDTGILMQPLIEGGDIVEPLHERVLGRVVASDVYIPTQTEPVVKAGTLLDEEWVEKLEKHGVDQVMVRSPITCQTRFGLCAKCYGRDLARGHLVNTGEAVGIIAAQSIGEPGTQLTMRTFHIGGAASRATAANNIQIKTKGVIRLHNIKTVTHENKNLVAVSRSGEVTIVDEFGRERERYKVPYGAVISAQDNSPVEAGQVIATWDPHTHPVISEVSGRLKFVDLIDGITMNRQTDELTGLSNIVIIDAKQRSAAGRDLRPMVKLVTDEGDDIYLAGTNVPAQYYLPVDAIVNFEDGSLVGIGDVIARIPQERSKTRDITGGLPRVADLFEARKPKDSAVMAEVSGLVNFGKETKGKRRLIINVSEDQCHEELIPKWRHISVFEGEHVERGEIIAEGALNPHDILRLLGVGALANYIVNEVQDVYRLQGVKINDKHIEVIVRQMLRKRVITFAGDSKFLVGEQVEESAMLQENDKLLAEGKQIARGTPILLGITKASLATESFISAASFQETTRVLTEAAVSGKVDELRGLKENVMVGRLIPAGTGYTYHQSRKAKRARAAAGGDSSATHTVTASDVEHALSEALNADNHEH

SEQ ID NO: 38 - protein, 1399 aa, Pseudomonas aeruginosa
MKDLLNLLKNQGQIEEFDAIRIGLASPEMIRSWSFGEVKKPETINYRTFKPERDGLFCAKIFGPVKDYECLCGKYKRLKHRGVICEKCGVEVALAKVRRERMGHIELASPVAHIWFLKSLPSRIGLLLDMTLRDIERVLYFESYVVIDPGMTTLEKGQLLNDEQYFEALEEFGDDFDARMGAEAVHELLNAIDLEHEIGRLREEIPQTNSETKIKKLSKRLKLMEAFQGSGNKPEWMVLTVLPVLPPDLRPLVPLDGGRFATSDLNDLYRRVINRNNRLKRLLDLAAPDIIVRNEKRMLQEAVDALLDNGRRGRAITGSNKRPLKSLADMIKGKQGRFRQNLLGKRVDYSGRSVITVGPTLRLHQCGLPKKMALELFKPFIFGKLEGRGMATTIKAAKKMVERELPEVWDVLAEVIREHPVLLNRAPTLHRLGIQAFEPVLIEGKAIQLHPLVCAAYNADFDGDQMAVHVPLTLEAQLEARALMMSTNNILSPANGEPIIVPSQDVVMGLYYMTREAINAKGEGMAFADLQEVDRAYRSGQASLHARVKVRINEKIKGEDGQLTANTRIVDTTVGRALLFQVVPAGLPFDVVNQSMKKKAISKLINHCYRVVGLKDTVIFADQLMYTGFAYSTISGVSIGVNDFVIPDEKARIINAATDEVKEIESQYASGLVTQGEKYNKVIDLWSKANDEVSKAMMANLSKEKVVDREGKEVDQESFNSMYMMADSGARGSAAQIRQLAGMRGLMAKPDGSIIETPITANFREGLNVLQYFISTHGARKGLADTALKTANSGYLTRRLVDVAQDLVVTEIDCGTEHGLLMSPHIEGGDVVEPLGERVLGRVIARDVFKPGSDEVIVPAGTLIDEKWVDFLEVMSVDEVVVRSPITCETRHGICAMCYGRDLARGHRVNIGEAVGVIAAQSIGEPGTQLTMRTFHIGGAASRTSAADNVQVKNGGTIRLHNLKHVVRADGALVAVSRSGELAVADDFGRERERYKLPYGAVISVKEGDKVDPGAIVAKWDPHTHPIVTEVDGTVAFVGMEEGITVKRQTDELTGLTNIEVMDPKDRPAAGKDIRPAVKLIDAAGKDLLLPGTDVPAQYFLPANALVNLTDGAKVSIGDVVARIPQETSKTRDITGGLPRVADLFEARRPKEPSILAEISGTISFGKETKGKRRLVITPNDGSDPYEELIPKWRHLNVFEGEQVNRGEVISDGPSNPHDILRLLGVSSLAKYIVNEIQDVYRLQGVKINDKHIETILRQMLRKVEVSESGDSSFIKGDQVELTQVLEENEQLGTEDKFPAKYERVLLGITKASLSTESFISAASFQETTRVLTEAAVTGKRDFLRGLKENVVVGRLIPAGTGLAYHSERKRQRDLGKPQRVSASEAEAALTEALNSSGN

SEQ ID NO: 39 - protein, 1401 aa, Vibrio cholerae
MKDLLNFLKAQHKTEEFDAIKIGLASPDMIRSWSFGEVKKPETINYRTFKPERDGLFCARIFGPVKDYECLCGKYKRLKHRGVICEKCGVEVTQTKVRRDRMGHIELASPVAHIWFLKSLPSRIGLLMDMPLRDIERVLYFEMYVVTEPGMTDLERGQMLTEEEYLDRLEEWGDEFTAKMGAEAIKDLLASMDLPAEAEQMREELDTTNSETKRKKLTKRLKLVEAFVASGNKPEWMILTVLPVLPPDLRPLVPLDGGRFATSDLNDLYRRVINRNNRLKRLLELAAPDIIVRNEKRMLQESVDALLDNGRRGRAITGSNKRPLKSLADMIKGKQGRFRQNLLGKRVDYSGRSVITVGPYLRLHQCGLPKKMALELFKPFIYSKLETRGLATTIKAAKKMVEREEAVVWDILDEVIREHPVLLNRAPTLHRLGIQAFEPVLIEGKAIQLHPLVCAAYNADFDGDQMAVHVPLTLEAQLEARTLMMSTNNILSPASGDPIIVPSQDVVLGLYYMTREKINAKGEGMYLTGPAEAEKAYRTKTAELHARVKVRITETIKHENGKLTTETKMIDTTVGRAMLWQIVPKGLPYSLVNQKLGKKQISNLLNEAYRKLGLKDTVIFADQIMYTGFAYAALSGVSVGIDDMVVPAAKYTEIAEAEEEVREIQEQFQSGLVTAGERYNKVIDIWASTNDRVAKAMMENLSSEQVINRQGEQEKQESFNSIYMMADSGARGSAAQIRQLAGMRGLMARPDGSIIETPITANFKEGLNVLQYFISTHGARKGLADTALKTANSGYLTRRLVDVAQDVVVTEHDCGTLEGVVMTPHIEGGDVKVALTELALGRVVSEDILKPGTDEVLIPRNTLLDEKWCKVINDNSVDQIKVRSVVTCDSDFGCCAQCYGRDLARGHLVNQGEAVGVIAAQSIGEPGTQLTMRTFHIGGAASTAAAENSIQAKNNGSVKLHNAKFVTNKDGKLVITSRASELTIIDEFGRTKEKHKLPYGSMLSKADGDAVAAGETVANWEAHTMPIITEVAGRVQFVDMIDGVTVSRQTDDLTGLSSSEVTEAAARPAAGKDMRPAIKLVDANGKDVLIPGTDMPAQYFLPGKAIVNLDDGAEVNVGDTLARIPQKSGGNKDITGGLPRVADLFEARKPKEPAILAEHSGTVSFGKETKGKRRLIITRDSGDTYEEMIPKHRQLNVFEGERIERGDVIADGPESPHDILRLRGIHAVTTYIANEVQEVYRLQGVKINDKHIETIVRQMLRKCTITFAGDSEFLPGETVEYSQVKIANRKLVEEGKEPARFERELLGITKASLATESFISAASFQETTRVLTEAAVSGKRDDLRGLKENVIVGRLIPAGTGFAYHQDRQAKRAQEQQGPSAEQATDNLAALLNAGFSSDDE

SEQ ID NO: 40 - protein, 1407 aa, Salmonella enterica
MKDLLKFLKAQTKTEEFDAIKIALASPDMIRSWSFGEVKKPETINYRTFKPERDGLFCARIFGPVKDYECLCGKYKRLKHRGVICEKCGVEVTQTKVRRERMGHIELASPTAHIWFLKSLPSRIGLLLDMPLRDIERVLYFESYVVIEGGMTNLERQQILTEEQYLDALEEFGDEFDAKMGAEAIQALLKSMDLEQECETLREELNETNSETKRKKLTKRIKLLEAFVQSGNKPEWMILTVLPVLPPDLRPLVPLDGGRFATSDLNDLYRRVINRNNRLKRLLDLAAPDIIVRNEKRMLQEAVDALLDNGRRGRAITGSNKRPLKSLADMIKGKQGRFRQNLLGKRVDYSGRSVITVGPYLRLHQCGLPKKMALELFKPFIYGKLELRGLATTIKAAKKMVEREEAVVWDILDEVIREHPVLLNRAPTLHRLGIQAFEPVLIEGKAIQLHPLVCAAYNADFDGDQMAVHVPLTLEAQLEARALMMSTNNILSPANGEPIIVPSQDVVLGLYYMTRDCVNAKGEGMVLTGPKEAERIYRAGLASLHARVKVRITEYEKDENGEFVAHTSLKDTTVGRAILWMIVPKGLPFSIVNQALGKKAISKMLNTCYRILGLKPTVIFADQTMYTGFAYAARSGASVGIDDMVIPEKKHEIISEAEAEVAEIQEQFQSGLVTAGERYNKVIDIWAAANDRVSKAMMDNLQTETVINRDGQEEQQVSFNSIYMMADSGARGSAAQIRQLAGMRGLMAKPDGSIIETPITANFREGLNVLQYFISTHGARKGLADTALKTANSGYLTRRLVDVAQDLVVTEDDCGTHEGILMTPVIEGGDVKEPLRDRVLGRVTAEDVLKPGTADILVPRNTLLHEQWCDLLEANSVDAVKVRSVVSCDTDFGVCAHCYGRDLARGHIINKGEAIGVIAAQSIGEPGTQLTMRTFHIGGAASRAAAESSIQVKNKGSIKLSNVKSVVNSSGKLVITSRNTELKLIDEFGRTKESYKVPYGAVMAKGDGEQVAGGETVANWDPHTMPVITEVSGFIRFTDMIDGQTITRQTDELTGLSSLVVLDSAERTTGGKDLRPALKIVDAQGNDVLIPGTDMPAQYFLPGKAIVQLEDGVQISSGDTLARIPQESGGTKDITGGLPRVADLFEARRPKEPAILAEIAGIVSFGKETKGKRRLVITPVDGSDPYEEMIPKWRQLNVFEGERVERGDVISDGPEAPHDILRLRGVHAVTRYIVNEVQDVYRLQGVKINDKHIEVIVRQMLRKATIESAGSSDFLEGEQVEYSRVKIANRELEANGKVGATFSRDLLGITKASLATESFISAASFQETTRVLTEAAVAGKRDELRGLKENVIVGRLIPAGTGYAYHQDRMRRRAAGEQPATPQVTAEDASASLAELLNAGLGGSDNE

SEQ ID NO: 41 - protein, 1300 aa, Actinomyces odontolyticus
MLDAKTFDSLKITLATGDDIAEWSHGEVKKPETINYRTLKPERDGLFGEQIFGPTRDWECACGKYKRVRYKGIVCEKCGVEVTRSRVRRERMGHIDLAAPVTHIWYFKGVPSRLGYVLNLAPKDLEKVIYFAAYMITEVDEKGRHEDLAELRAELEVQKKQMENNRDATINDFAEQLESDMAALEKDGASQAERERARKQGEREMAKIRRRFDGDIEGLEAVWERFKDLKVGDLEGDERLYRAMVARYGTYFKGDMGAAAIQKRLETFDLEAEVAALRQTIGSDSGPRKARAIKRLKVINAFVATGNSPASMVLTKIPVIPPDLRPMVQLDGGRFATSDLNDLYRRVINRNTRLKRLLELGAPEIIVNNEKRMLQESVDALFDNGRRGRPVAGPGNRPLKSISDMLKGKQGRFRQNLLGKRVDYSGRSVIVVGPQLQLHQCGLPKQMALELFKPFVMKRLVEKNYAQNVKAAKRKVERQRPEVWDVLDDVIREHPVLLNRAPTLHRLGIQAFEPQLIEGKAIQLHPLACGAFNADFDGDQMAVHLPLGAEAQAEARILMLSTNNILKPSDGRPVAMPSQDMIIGLFHLTSTPDPSVPVEKDEDGNPVIPYFSSQAEAQMAYDAGNLHLNATARIRFADGTVPPEGWEAPEGWEPGDELILETSLGRAIFNEQLPTDYPFINEVVGKKQLGNIVNTLTQRYPNVLVADCLDALKSAGFHWSTWSGITIAFSDIQASPRKREILARYEAKAAEIVEQFETGIILEETRYEELVKLWLQCTEEVADDMRANFDERNTVYRMVNSGARGNWSQVQQIAGMRGLVSDPKQKLIEQPIKANYREGLTVLEYFIATHGARKGLVDTALRTAESGYLTRRLVDVSQDVIVREGDCGTRAGLKIDIAHKNEFGEWEASETIETTAYARNLARDAVNEAGEVVMPAGTDLGDDQLAELVAAGVEQIVCRSVLTCESQVGTCAACYGRSLATGKQVDIGEAVGIIAAQSIGEPGTQLTMRTFHTGGAASAADITQGLPRVQELFEARSPKVEAKMNEAAGRVHIDDEDPSARKVVITRDDGKEDLVIEVSRRQKLLVSEGQHIEAGTPLTEGQLDPKEILRIMGRNVSQKMLVDEVQKVYRDQGVGIHAKHIEVIVRQMLRRVTILEPGDTTFMPGELVDRMAYLTQNRRVAAEGGQPASGRQMLMGITKASLATDSWLSAASFQETTKVLTEAAMNGKSDSLVGLKENVILGKLIPAGTGLSRYNDVIVEPTAEAMANSNYSEADFGDGSVSEDFLDALGAIDFGMNFRE

SEQ ID NO: 42 - protein, 1299 aa, Streptomyces coelicolor
MLDVNFFDELRIGLATADDIRQWSHGEVKKPETINYRTLKPEKDGLFCEKIFGPTRDWECYCGKYKRVRFKGIICERCGVEVTRAKVRRERMGHIELAAPVTHIWYFKGVPSRLGYLLDLAPKDLEKVIYFAAYMITFVDEERRTRDLPSLEAHVSVERQQIEQRRDSDLEARAKKLETDLAELEAEGAKADVRRKVREGAEREMKQLRDRAQREIDRLDEVWNRFKNLKVQDLEGDELLYRELRDRFGTYFDGSMGAAALQKRLESFDLDEEAERLREIIRTGKGQKKTRALKRLKVVSAFLQTSNSPKGMVLDCVPVIPPDLRPMVQLDGGRFATSDLNDLYRRVINRNNRLKRLLDLGAPEIIVNNEKRMLQEAVDALFDNGRRGRPVTGPGNRPLKSLSDMLKGKQGRFRQNLLGKRVDYSARSVIVVGPQLKLHQCGLPKAMALELFKPFVMKRLVDLNHAQNIKSAKRMVERGRTVVYDVLEEVIAEHPVLLNRAPTLHRLGIQAFEPQLVEGKAIQIHPLVCTAFNADFDGDQMAVHLPLSAEAQAEARILMLSSNNILKPADGRPVTMPTQDMVLGLFFLTTDSEGRSPKGEGRAFGSSAEAIMAFDAGDLTLQAKIDIRFPVGTIPPRGFEPPAREEGEPEWQQGDTFTLKTTLGRALFNELLPEDYPFVDYEVGKKQLSEIVNDLAERYPKVIVAATLDNLKAAGFFWATRSGVTVAISDIVVPDAKKEIVKGYEGQDEKVQKQYERGLITKEERTQELIAIWTKATNEVAEAMNDNFPKTNPVSMMVNSGARGNMMQMRQIAGMRGLVSNAKNETIPRPIKASFREGLSVLEYFISTHGARKGLADTALRTADSGYLTRRLVDVSQDVIIREEDCGTERGLKLPIATRDADGTLRKAEDVETSVYARMLAEDVVIDGKVIAPANVDLGDVLIDALVAHGVEEVKTRSILTCESQVGTCAMCYGRSLATGKLVDIGEAVGIIAAQSIGEPGTQLTMRTFHTGGVAGDDITQGLPRVVELFEARTPKGVAPISEASGRVRIEETEKTKKIVVTPDDGSDETAFPISKRARLLVGEGDHVEVGQKLTVGATNPHDVLRILGQRAVQVHLVGEVQKVYNSQGVSIHDKHIEIIIRQMLRRVTIIESGDAELLPGELVERTKFETENRRVVQEGGHPASGRPQLMGITKASLATESWLSAASFQETTRVLTDAAINAKSDSLIGLKENVIIGKLIPAGTGLSRYRNIRVEPTEEAKAAMYSAVGYDDIDYSPFGTGSGQAVPLEDYDYGPYNQ

SEQ ID NO: 43 - protein, 1336 aa, Corynebacterium diphtheriae
MIDVNFFDELRIGLATADDIRRWSKGEVKKPETINYRTLKPEKDGLFCERIFGPTRDWECACGKYKRVRYKGIICERCGVEVTKSKVRRERMGHIELAAPVTHIWYFKGVPSRLGYLLDLAPKDLERIIYFAANIITSVDDEARHADQTTLEAEMLLEKKDVEADMESEIAERAAKLEEDLAELEAAGAKADARNKVKKAAEKEMQHIRERAEREIDRLEEIWQTFIKLAPKQMIIDETIYEELVDRYEDYFTGGMGAEAIQTLIRNFDLDSEAEELREIINNGKGQKKMRALKRLKVVAAFQRSGNDPAGMVLDCIPVIPPELRPMVQLDGGRFATSDLNDLYRRVINRNNRLKRMIELGAPEIIVNNEKRMLQESVDALFDNGRRGRPVTGPGNRPLKSLSDLLKGKQGRFRQNLLGKRVDYSGRSVIIVGPQLKLHECGLPKLMALELFKPFVMKRLVENDYAQNIKSAKRMVERQRPEVWDVLEEAISEHPVMLNRAPTLHRLGIQAFEPKLVEGKAIQLHPLACEAFNADFDGDQMAVHLPLSAEAQAEARILMLASNNILSPASGKPLAMPRLDMVTGLYYLTMDKNENEIGGQGAYASATEEGPAQGVYSSYAEAIMARDRGVLGLQAKIKVRISHLRPPVDIEAEQFPEGWNKGDVWLADTTLGRIMFNELLPWNYPYLEGVMVRKGGGTGKIMLGDVINDLAATYPMITVAQTMDKMKDAGFYWATRSGVTITMSDVLVLPNKEEILDRYEAEARKIERKYWEQGALTERERYDRLVELWKDATDEVGNAVEKLYPDDNPIPMIVKSGAAGNMRQIWTLAGMKGMVVNSKGDYITRPIKTSFREGLSVLEYFNNSHGSRKGLADTALRTADSGYLTRRLVDVAQDVIVREDDCGTKQGIRVPVAVEVKDAEGNVTGYTGHSLIETSVAGRVAATAVKDAEGNVMVEPGENLTDQLIDELIAAGVKEVKVRSVLTCQTPTGVCAKCYGKSMATGKLVDIGEAVGIVAAQSIGEPGTQLTMRTFHQGGVGGDITGGLPRVQELFEARVPKNRAPIASVAGTVHLDDEGNFYTLTINPDDGSDVVVYEKLSKRQGLATVRVPMESNPGAMIERTLAEGDHVEVGDRLLRGPADPHDVLEVLGRRGVEQHLVDEVQDVYRAQGVAIHDKHIEIIIRQMLRRGTVIESGSTEFLPGTLVDLSEAKAANAEALANGGQPAELRSEIMGITKASLATESWLSAASFQETTRVLTDAAINKRSDKLIGLKENVIIGKLIPAGTGISRYRNISVKPTEAARNAAYSIPTYGDSIYGDDGYGEFTGASVPLDEAYDL

SEQ ID NO: 44 - protein, 1316 aa, Mycobacterium tuberculosis
MLDVNFFDELRIGLATAEDIRQWSYGEVKKPETINYRTLKPEKDGLFCEKIFGPTRDWECYCGKYKRVRFKGIICERCGVEVTRAKVRRERMGHIELAAPVTHIWYFKGVPSRLGYLLDLAPKDLEKIIYFAAYVITSVDEEMRHNELSTLEAEMAVERKAVEDQRDGELEARAQKLEADLAELEAEGAKADARRKVRDGGEREMRQIRDRAQRELDRLEDIWSTFTKLAPKQLIVDENLYRELVDRYGEYFTGAMGAESIQKLIENFDIDAEAESLRDVIRNGKGQKKLRALKRLKVVAAFQQSGNSPMGMVLDAVPVIPPELRPMVQLDGGRFATSDLNDLYRRVINRNNRLKRLIDLGAPEIIVNNEKRMLQESVDALFDNGRRGRPVTGPGNRPLKSLSDLLKGKQGRFRQNLLGKRVDYSGRSVIVVGPQLKLHQCGLPKLMALELFKPFVMKRLVDLNHAQNIKSAKRMVERQRPQVWDVLEEVIAEHPVLLNRAPTLHRLGIQAFEPMLVEGKAIQLHPLVCEAFNADFDGDQMAVHLPLSAEAQAEARILMLSSNNILSPASGRPLAMPRLDMVTGLYYLTTEVPGDTGEYQPASGDHPETGVYSSPAEAIMAADRGVLSVRAKIKVRLTQLRPPVEIEAELFGHSGWQPGDAWMAETTLGRVMFNELLPLGYPFVNKQMHKKVQAAIINDLAERYPMIVVAQTVDKLKDAGFYWATRSGVTVSMADVLVPPRKKEILDHYEERADKVEKQFQRGALNHDERNEALVEIWKEATDEVGQALREHYPDDNPIITIVDSGATGNFTQTRTLAGMKGLVTNPKGEFIPRPVKSSFREGLTVLEYFINTHGARKGLADTALRTADSGYLTRRLVDVSQDVIVREHDCQTERGIVVELAERAPDGTLIRDPYIETSAYARTLGTDAVDEAGNVIVERGQDLGDPEIDALLAAGITQVKVRSVLTCATSTGVCATCYGRSMATGKLVDIGEAVGIVAAQSIGEPGTQLTMRTFHQGGVGEDITGGLPRVQELFEARVPRGKAPIADVTGRVRLEDGERFYKITIVPDDGGEEVVYDKISKRQRLRVFKHEDGSERVLSDGDHVEVGQQLMEGSADPHEVLRVQGPREVQIHLVREVQEVYRAQGVSIHDKHIEVIVRQMLRRVTIIDSGSTEFLPGSLIDRAEFEAENRRVVAEGGEPAAGRPVLMGITKASLATDSWLSAASFQETTRVLTDAAINCRSDKLNGLKENVIIGKLIPAGTGINRYRNIAVQPTEEARAAAYTIPSYEDQYYSPDFGAATGAAVPLDDYGYSDYR

SEQ ID NO: 45 - protein, 1319 aa, Rhodococcus equi
MLDVNFFDELRIGLATAEDIRNWSYGEVKKPETINYRTLKPEKDGLFCEKIFGPTRDWECYCGKYKRVRFKGIICERCGVEVTRAKVRRERMGHIELAAPVTHIWYFKGVPSRLGYLLDLAPKDLEKIIYFAAYVIVGVDEELRHNELSTLEAEMEVEKKTVADQRDADLEARAQKLEADIAELEAEGAKSDVRRKVKDGGEREMRQLRDRAQRELDRLDEIWTTFTKLSVKQLIVDESLYRELVDRYGEYFTGAMGAESIQKLMENFDIEAEAESLRETIRSGKGQKKLRALKRLKVVAAFQQSGNSPMGMVLDAVPVIPPELRPMVQLDGGRFATSDLNDLYRRVINRNNRLKRLIDLGAPEIIVNNEKRMLQESVDALFDNGRRGRPVTGPGNRPLKSLSDLLKGKQGRFRQNLLGKRVDYSGRSVIVVGPQLKLHQCGLPKLMALELFKPFVMKRLVDLNHAQNIKSAKRMVERQRPQVWDVLEEVINEHPVLLNRAPTLHRLGIQAFEPQLVEGKAIQLHPLVCEAFNADFDGDQMAVHLPLSAEAQAEARILMLSSNNILSPASGRPLAMPRLDMVTGLFHLTREVEGAIGAYQPAADGQPEQGVYSSPAEAQMAVDRGVLSVQAKIKVRLTHQRPPREIEAELFPEGWNFGDGWMVETTLGRVMFNDLLPADYPFINEQMPKKRQATIINDLAERYPMIVVAQTVDKMKDTGFYWATRSGVTVSISDVLVPPEKAQIMEQFEAQADQIEKKYQRGALNHTERNSALVKIWSEATDEVGKAMEAHFPDDNPIPMIVKSGAAGNMTQVRSLAGMKGLVTNPKGEFIPRPIKSSFKEGLTVLEYFINTHGARKGLADTALRTADSGYLTRRLVDVSQDVIVREVDCGTERGILTTIAEKAADGTMIRDAHVETSTYARTLAADAIDENGNVVVERGHDLGDPAIDALLAAGITQVKVRSVLTCTTATGVCATCYGRSMATGKLVDIGEAVGIVAAQSIGEPGTQLTMRTFHQGGAAGAADITGGLPRVQELFEARVPKGKAPITEVSGRVQLDDDDRFYKITVVPDDGGEEVVYDKLSKRQRLRVFKHDDGSERLLSDGDHVDVGQQLLEGAADPHDVLRVMGPRQVQIHLVNEVQEVYRSQGVSIHDKHIEVIVRQMLRRVTIIDSGSTEFLPGSLVERAEFEASNRRVVAEGGEPAAGRPVLMGITKASLATDSWLSAASFQETTRVLTDAAINCRSDKLIGLKENVIIGKLIPAGTGINRYRNIQVQPTEEARAAAYAVPSYDDQYYSPEGFGTGTGAAVPLDDYGFGSDYR

SEQ ID NO: 46 - protein, 1396 aa, Chlamydia trachomatis
MFREGSRDDAALVKEGLFDKLEIGIASDVTIRDKWSCGEIKKPETINYRTFKPEKGGLFCEKIFGPTKDWECYCGKYKKIKHKGIVCDRCGVEVTLSKVRRERMAHIELAVPIVHIWFFKTTPSRIGNVLGMTASDLERVIYYEEYVVIDPGNTDLVKKQLLNDAKYREVVEKWGKDAFVAKMGGEAVYDLLKSEDLESLLGELKERLRKTKSQQARMKLAKRLKIVEGFVSSSNRPEWMVLKNIPVVPPDLRPLVPLDGGRFATSDLNDLYRRVINRNNRLKAILRLKTPEVIVRNEKRMLQEAVDALFDNGRHGHPVMGAGNRPLKSLSEMLKGKNGRFRQNLLGKRVDYSGRSVIIVGPELKFNQCGLPKEMALELFEPFIIKRLKDQGSVYTIRSAKKMIQRGAPEVWDVLEEIIKGHPVLLNRAPTLHRLGIQAFEPVLIEGKAIRVHPLVCAAFNADFDGDQMAVHVPLSIEAQLEAKVLMMAPDNIFLPSSGKPVATPSKDMTLGIYYLMADPTYFPEEHGGKTKAFKDEVEVLRALNAGGFILKDEICGSRRDETGRGIHIHEKIKVRIDGQIIETTPGRVFFNTIVPKELGFQNYSMPSKRISELILQCYKKVGLEATVRFLDDLKELGFVQSTKAAISMGLKDVKIPEIKKEILKDAYDKVAVVKKQYEDGIITDGERHSKTISIWTEVSDLLSNALYSEIKKQTNSKHNPLFLMIDSGARGNKSQLKQLGALRGLMAKPNGAIIESPITSNFREGLTVLEYSISSHGARKGLADTALKTADSGYLTRRLVDVAQDVIITERDCGTLNHIEVSTIRQGSEELLPLKDRVYGRTVSENIYQPGDKSNVLAYAGDVLTSAQAEAIDDAGIESVKIRSTLTCESRRGVCAKCYGLNLANGRLIGLGEAVGIIAAQSIGEPGTQLTMRTFHLGGIAATSSTPEIVAECDGILVYLDLRVVVDQEGNNLVLNKMGALHLVQDEGRSLSEYKKLLSTKSIESLATFPVELGAKILVNDGAAVAAGQRIAEVELHNIPIICDKPGFVHYEDLVEGVSTEKVTNKNTGLVELIVKQHRGELHPQIAIYADANMKELVGTYAIPSGAIISVEEGQRIAPGMLLARLPRGAIKTKDITGGLPRVAELVEARKPEDAADIAKIDGVVDFKGIQKNKRILVVRDEITGMEEEHLISLTKHLIVQRGDSVIKGQQLTDGLVVPHEILEICGVRELQKYLVNEVQEVYRLQGVDINDKHVEIIVRQMLQKVRITDPGDTTLLFGEDVDKKEFYEENRRTEEDGGKPAQAVPVLLGITKASLGTESFISAASFQDTTRVLTDAACSSKTDYLLGFKENVIMGHMIPGGTGFDTHKRIKQHLEKEQEDLVFDFDSEFESVAG

SEQ ID NO: 47 - protein, 1178 aa, Clostridium botulinum
MFELNNFDALQIGLASPEKIREWSRGEVKKPETINYRTLKPERDGLFCERIFGPMKDWECHCGKYKRIRYKGIVCDRCGVEVTKAKVRRERMGHIELAAPVSHIWYFKGIPSRMGLILDMSPRALEKVLYFASYVVLDPKETPLLKKQLLNEKEYRESIDKYGDDSFVAAMGAEAVKTLLDEIDLEQSSIELKEELKTSTGQKKIRIIRRLEVVESFRKSGNRPDWMVIDVIPVIPPDLRPMVQLDGGRFATSDLNDLYRRVINRNNRLKKLLDLGAPDIIVRNEKRMLQEAVDALIDNGRRGRPVTGPGNRPLKSLSDMLKGKQGRFRQNLLGKRVDYSGRSVIVVGPELKMYQCGLPKEMALELFKPFVMKKLVQNGLAHNIKSAKRMVERVQPQVWDVLEEVISDHPVLLNRAPTLHRLGIQAFQPVLVEGRAIKLHPLVCTAYNADFDGDQMAVHVPLSVEAQAEARFLMLAAHNILKPSDGKPVSVPTQDMVLGSYYLTMDKDGVKGEGKVFSCPEEVLMAYQCKAVDIHAKIKVRLKKVIDGETIEGIIETTPGKIIFNESIPQDLGYIDRTVPENKLKLEVDFLVSKKTLGGIINRCYMKHGATKTSIMLDKIKAKGYHYSTIGAITISTSDMVVPEAKRELLQNTEKQVEKIQKMYRRGFISEEERYEKVIDLWTKTTEDVANALMASLDSFNPIYMMADSGARGSKSQIKQLAGMRGLMANPSGKIIELPIKASFREGLDVLEYFISTHGARKGNADTALKTADSGYLTRRLVDVSQDVIVRQEDCGTEEGYEVSEIKEGNEVIEPLVERLSGRYPSEDIINPTTGEVIVKRNTYMNEDIAKKVSDAGIKKVKIRSVFTCKSKHGVCARCYGMNMATSQKIHIGEAVGIVAAQSIGEPGTQLTMRTFHTGGVAGADITQGLPRVEELFEARKPKGLAIVSEVSGTVKMEETKKKRTIIVVTDDGEEVSYDIPFGSRIKVKNGDIISAGDEITEGSINPHDILRIKGVDGVKNYLLSEVQKVYRLQGVDINDKHLEVVIRQMTRKIKIEDSGDTELLPGTMIDVFDFEEANREILEKGGEPAVGRIALLGITKAALATDSFLSAASFQETTRVLTDAAIKGKIDPLLGLKENVIIGKLIPAGTGMTRYRSIQINTDDENIEEDSMDSIEV

SEQ ID NO: 48 - protein, 1199 aa, Bacillus subtilis
MLDVNNFEYMNIGLASPDKIRSWSFGEVKKPETINYRTLKPEKDGLFCERIFGPTKDWECHCGKYKRVRYKGVVCDRCGVEVTRAKVRRERMGHIELAAPVSHIWYFKGIPSRMGLVLDMSPRALEEVIYFASYVVTDPANTPLEKKQLLSEKEYRAYLDKYGNKFQASMGAEAIHKLLQDIDLVKEVDMLKEELKTSQGQRRTRAIKRLEVLEAFRNSGNKPSWMILDVLPVIPPELRPMVQLDGGRFATSDLNDLYRRVINRNNRLKRLLDLGAPSIIVQNEKRMLQEAVDALIDNGRRGRPVTGPGNRPLKSLSHMLKGKQGRFRQNLLGKRVDYSGRSVIVVGPHLKMYQCGLPKEMALELFKPFVMKELVEKGLAHNIKSAKRKIERVQPEVWDVLESVIKEHPVLLNRAPTLHRLGIQAFEPTLVEGRAIRLHPLVCTAYNADFDGDQMAVHVPLSAEAQAEARILMLAAQNILNPKDGKPVVTPSQDMVLGNYYLTLERAGAVGEGMVFKNTDEALLAYQNGYVHLHTRVAVAANSLKNVTFTEEQRSKLLITTVGKLVFNEILPESFPYMNEPTKSNIEEKTPDRFFLEKGADVKAVIAQQPINAPFKKGILGKIIAEIFKRFHITETSKMLDRMKNLGFKYSTKAGITVGVSDIVVLDDKQEILEEAQSKVDNVMKQFRRGLITEEERYERVISIWSAAKDVIQGKLMKSLDELNPIYMMSDSGARGNASNFTQLAGMRGLMANPAGRIIELPIKSSFREGLTVLEYFISTHGARKGLADTALKTADSGYLTRRLVDVAQDVIIRETDCGTDRGILAKPLKEGTETIERLEERLIGRFARKQVKHPETGEVLVNENELIDEDKALEIVEAGIEEVWIRSAFTCNTPHGVCKRCYGRNLATGSDVEVGEAVGIIAAQSIGEPGTQLTMRTFHTGGVAGDDITQGLPRIQELFEARNPKGQATITEIDGTVVEINEVRDKQQEIVVQGAVETRSYTAPYNSRLKVAEGDKITRGQVLTEGSIDPKELLKVTDLTTVQEYLLHEVQKVYRMQGVEIGDKHVEVMVRQMLRKVRVIDAGDTDVLPGTLLDIHQFTEANKKVLLEGNRPATGRPVLLGITKASLETDSFLSAASFQETTRVLTDAAIKGKRDELLGLKENVIIGKLVPAGTGMMKYRKVKPVSNVQPTDDMVPVE

SEQ ID NO: 49 - protein, 1225 aa, Streptococcus pneumoniae
MVDVNRFKSMQITLASPSKVRSWSYGEVKKPETINYRTLKPEREGLFDEVIFGPTKDWECACGKYKRIRYRGIVCDRCGVEVTRTKVRRERMGHIELKAPVSHIWYFKGIPSRMGLTLDMSPRALEEVIYFAAYVVIDPKDTPLEHKSIMTEREYRERLREYGYGSFVAKMGAEAIQDLLKQVDLEKEIAELKEELKTATGQKRVKAIRRLDVLDAFYKSGNKPEWMILNILPVIPPDLRPMLQLDGGRFASSDLNDLYRRVINRNNRLARLLELNAPGIIVQNEKRMLQEAVDALIDNGRRGRPITGPGSRPLKSLSHMLKGKQGRFRQNLLGKRVDFSGRSVIAVGPTLKMYQCGVPREMAIELFKPFVMREIVARDIVQNVKAAKRLVERGDERIWDILEEVIKEHPVLLNRAPTLHRLGIQAFEPVLIDGKALRLHPLVCEAYNADFDGDQMAIHVPLSEEAQAEARILMLAAEHILNPKDGKPVVTPSQDMVLGNYYLTMEEAGREGEGMVFKDRDEAVMAYRNGYVHLHSRVGIATDSLNKPWTEEQRHKVLLTTVGKILFNDIMPEGLPYLQEPNNANLTEGVPAKYFLPLGGDIKEAISNLELNPPFKKKNLGNIIAEIFKRFRTTETSALLDRMKNLGYHHSTLAGLTVGIADIPVVDDKAEIIEESHKRVEQITKQFRRGMITDDERYNAVTAEWRAAREKLEKRLIANQDPKNPIVMMMDSGARGNISNFSQLAGMRGLMAAPNGRIMELPILSNFREGLSVLEMFFSTHGARKGMTDTALKTADSGYLTRRLVDVAQDVIIREDDCGTDRGLLIRSIAEGKEMIESLEERLNGRYTKKTVKHPETGAVIIGPNELITEDKAREIVNAGVEEVTIRSVFTCNTRHGVCRHCYGINLATGDAVEVGEAVGTIAAQSIGEPGTQLTMRTFHTGGVASNTDITQGLPRVQEIFEARNPKGEAVITEVKGQVTAIEEDASTRTKKVFVKGETGEGEYVVPFTARMRVEVGGQVARGAALTEGSIQPKRLLAVRDVLSVETYLLGEVQKVYRSQGVEIGDKHIEVMVRQMIRKVRVMDPGDTDLLMGTLMDINDFTDANKDVLIAGGVPATGRPVLMGITKASLETNSFLSAASFQETTRVLTDAAIRGKKDHLLGLKENVIIGKIIPAGTGMARYRNLEPHAVNEEEYLNPPVEEEGNEETTEVVVDTAVETVEETVE

SEQ ID NO: 50 - protein, 1217 aa, Enterococcus faecalis
MIDVNKFESMQIGLASPEKIRSWSYGEVKKPETINYRTLKPEREGLFCERIFGPTKDWECACGKYKRIRYKGIVCDRCGVEVTRSKVRRERMGHIELAAPVSHIWYFKGIPSRMGLVLDMSPRALEEVIYFASYVVIEPGDTTLEKKQLLTEREYREKREQYGQAFKAAMGAEAVKQLLDNVDLDGEVAQLKEELKTASGQKRTRAIRRLDILEAFRASGNQPSWMVMDVIPVIPPDLRPMVQLEGGRFATSDLNDLYRRVINRNNRLKRLLDLNAPSIIVQNEKRMLQEAVDALIDNGRRGRPVTGPGNRPLKSLSHMLKGKQGRFRQNLLGKRVDYSGRSVIVVGPFLKMYQCGLPKEMAIELFKPFVMRELVQREIATNIKNAKRKIERGEDEVWDILEEVIQEHPVLLNRAPTLHRLGIQAFEPVLVEGRAIRLHPLVCEAYNADFDGDQMAVHVPLNEEAQAEARMLMLAAQNILNPKDGKPVVTPSQDMVLGNYYLTMEEEGREGEGMIFRDMNEAVLAWQNGYVHLHSRIGVQTTLLGDKPFTDWQKERILITTVGKIIFNEIMPVEFPYLNEPTDYNLTVQTPDKYFVEAGTDIPAHIKEQELVLPFKKKNLGNIIAEVFKRFHITETSKMLDRMKDLGYKHSTYAGMTVGIADIMVLHEKQAIIDAAHKQVETITKQFRRGLITDDERYERVIGVWNGAKDEIQQKLIESMEARNPIFMMSDSGARGNISNFTQLAGMRGLMAAPNGRIMELPIISNFREGLSVLEMFISTHGARKGMTDTALKTADSGYLTRRLVDVAQDVIIREDDCGTDRGLEIEAIREGNEIIEPLDERLLGRYTRKSVVHPETGAIIIGADQLITEDLAREIVDAGIEKVTIRSVFTCNTKHGVCKHCYGRNLATGSDVEVGEAVGTIAAQSIGEPGTQLTMRTFHTGGVAGDDITQGLPRIQEIFEARNPKGQAVITEVTGEVIDISEDPATRQKEVTIKGKTDTRTYTVPYTARMKVAEGDIIHRGAPLTEGSIDPKQLLQVRDVLSVENYLLREVQRVYRMQGVEIGDKHIEVMVRQMLRKIRVMDPGDTEILPGTLMDIAEFKDRNYDTLVAGGVPATSRPVLLGITKASLETNSFLSAASFQETTRVLTDAAIRGKKDPLLGLKENVIIGKIIPAGTGMARYRNMEPKEVGVASENVYSISDIEAQMAAEDAMKNINK

SEQ ID NO: 51 - protein, 1215 aa, Lactobacillus brevis
MVDVNKFESMQIGLASPDKIRSWSYGEVKKPETINYRTLKPEKDGLFDERIFGPTKDWECACGKYKRIRYKGVVCDRCGVEVTRSKVRRERMGHIELAAPVTHIWYFKGIPSRMGLVLDMSPRALEEIIYFASYVVLDPGNTPLEKKQLLSERDYRDKLLEYGSDAFKAEMGAEAIKKLLMSVDLDKEVTELKEELKEATGQKRTRAVRRLDILEAFVMSGNRPEWMVMDAIPVIPPDLRPMVQLEGGRFATSDLNDLYRRVINRNSRLKRLLDLNAPGIIVQNEKRMLQEAVDALIDNGRRGRPVAGPGNRPLKSLSHMLKGKQGRFRQNLLGKRVDYSGRSVIDVGPSLKFNQMGLPVPMALELFRPFIMKELVARGLASNIKNAKRQIDREDDDVFNVLEDVIKEHPVLLNRAPTLHRLGIQAFEPVLVSGKAMRLHPLACEAYNADFDGDQMAIHVPLSDEAQAEARLLMLAAHHILAPASGKPVVAPSQDMVIGNYYLTMEEANREGEGMIFTDLDEATLAYRNGIVHWHTRVGVQVTSMPDKPFTDEQRSKIMVTTVGKLIFNNILPKSFPYLNEPTSTNLNGYVPDKYFLEPGEDIHDYLQNAEIIPPFKKGFLSDIIAAVYQQYKVTATSELLDRIKDLGYNESTKSGLTVGMVDVTDLKEKPEIIAAAHKQVSTVTKQFRRGLITDHERYERVIGIWNDAKDEIQNALIHSFDQQNPIFMMSDSGARGNISNFTQLAGMRGLMAAPSGDIMELPITSNFREGLTVMEMFISTHGARKGMTDTALKTANSGYLTRRLVDVAQDVIIREKDCGTDRGLKIRAITDGNEMIEPLYDRILGRYTQKTVYDPQTGDVIVPKNQMIVEDTAQQIVDAGVEEVTIRSAFTCNTEHGVCEHCYGRNMATGDEVEVGEAVGTVAAQSIGEPGTQLTMRNFHTGGVAGNEDITQGLPRVQELFESRNPKGKAEITEVTGTVESIEENPAERTKEITIKGEADTRSYTLPITARMRVSEGDFIHRGGALNYGSVDPKELLRVRDVLSTETYILGEVQRVYRMQGVAISDKHVEIMVRQMLRKVRIMDPGDTDVLPGTLMDIQDFRRANYQTLIDGGIAATARPVILGITKAALETNSFLSAASFQETTRVLTDAAIRGKNDPLVGLKENVIIGKIIPAGTGMPDYRQIKPKEVGGTSTEGVYSISDLEKQMQEDSQA